European Patent Application EP 4 717 772 A9, published August 5, 2026. Title: USE OF REGULATOR OF ITPRIPL1 IN PREPARATION OF DRUG THAT REGULATES IMMUNE RESPONSES OR FIGHTS TUMORS. Applicant: FUDAN UNIVERSITY. Application EP 25222833.3, filed October 29, 2021. The sequence listing filed with the application follows.

SEQUENCE LISTING (99 sequences)

SEQ ID NO: 1 - protein, 79 aa, Homo sapiens
HPLMVSDRMDLDTLARSRQLEKRMSEEMRLLEMEFEERKRAAEQRQKAENFWTGDTSSDQLVLGKKDMGWPFQADGQEG

SEQ ID NO: 2 - protein, 54 aa, Homo sapiens
DRMDLDTLARSRQLEKRMSEEMRLLEMEFEERKRAAEQRQKAENFWTGDTSSDQ

SEQ ID NO: 3 - protein, 42 aa, Homo sapiens
MDLDTLARSRQLEKRMSEEMRLLEMEFEERKRAAEQRQKAEN

SEQ ID NO: 4 - protein, 103 aa, Homo sapiens
MNVDAEASMAVISLLFLAVMYVVHHPLMVSDRMDLDTLARSRQLEKRMSEEMRLLEMEFEERKRAAEQRQKAENFWTGDTSSDQLVLGKKDMGWPFQADGQEG

SEQ ID NO: 5 - protein, 310 aa, Homo sapiens
HPLMVSDRMDLDTLARSRQLEKRMSEEMRLLEMEFEERKRAAEQRQKAENFWTGDTSSDQLVLGKKDMGWPFQADGQEGPKSCDKTHTCPPCPAPELLGGPSVFLFPPKPKDTLMISRTPEVTCVVVDVSHEDPEVKFNWYVDGVEVHNAKTKPREEQYNSTYRVVSVLTVLHQDWLNGKEYKCKVSNKALPAPIEKTISKAKGQPREPQVYTLPPSRDELTKNQVSLTCLVKGFYPSDIAVEWESNGQPENNYKTTPPVLDSDGSFFLYSKLTVDKSRWQQGNVFSCSVMHEALHNHYTQKSLSLSPGK

SEQ ID NO: 6 - protein, 285 aa, Homo sapiens
DRMDLDTLARSRQLEKRMSEEMRLLEMEFEERKRAAEQRQKAENFWTGDTSSDQPKSCDKTHTCPPCPAPELLGGPSVFLFPPKPKDTLMISRTPEVTCVVVDVSHEDPEVKFNWYVDGVEVHNAKTKPREEQYNSTYRVVSVLTVLHQDWLNGKEYKCKVSNKALPAPIEKTISKAKGQPREPQVYTLPPSRDELTKNQVSLTCLVKGFYPSDIAVEWESNGQPENNYKTTPPVLDSDGSFFLYSKLTVDKSRWQQGNVFSCSVMHEALHNHYTQKSLSLSPGK

SEQ ID NO: 7 - protein, 273 aa, Homo sapiens
MDLDTLARSRQLEKRMSEEMRLLEMEFEERKRAAEQRQKAENPKSCDKTHTCPPCPAPELLGGPSVFLFPPKPKDTLMISRTPEVTCVVVDVSHEDPEVKFNWYVDGVEVHNAKTKPREEQYNSTYRVVSVLTVLHQDWLNGKEYKCKVSNKALPAPIEKTISKAKGQPREPQVYTLPPSRDELTKNQVSLTCLVKGFYPSDIAVEWESNGQPENNYKTTPPVLDSDGSFFLYSKLTVDKSRWQQGNVFSCSVMHEALHNHYTQKSLSLSPGK

SEQ ID NO: 8 - DNA, 1710 bp, Homo sapiens
  source 1..1710: mol_type = genomic DNA
gaattcgccaccatgaatgttgatgcagaggcctccatggctgtgataagcctgctgttcttggcagtgatgtatgttgttcaccaccctctgatggtcagtgatcggatggacctggacacattagccaggagtcggcagctggagaagcgaatgagtgaggagatgcgcctgctagagatggagtttgaagagagaaagcgagccgctgagcagaggcagaaggcagagaacttctggacaggagacacatccagtgaccagttagtgctggggaagaaagacatggggtggccgttccaggccgatggccaggaagggcctctgggctggatgctgggaaacctgtggaacactggcctcttttgcctttttctcgtctttgagctcctgcgacagaacatgcagcatgaaccggcctttgattccagcagtgaggaggaggaggaggaagtccgtgttgtccctgtcacctcttacaactggcttactgacttcccctcccaggaggccctggactccttttacaaacactatgtccaaaatgccatccgtgacctgccctgcacctgtgagtttgtggagagttttgtggatgatctcattgaggcctgtcgggtgctcagccgccaagaggctcacccacaattggaagactgcctgggcatcggggctgcctttgagaaatggggaaccctccatgagacccagaaatttgatatcctggtgcccattgtccccccacagggcaccatgtttgtcctggagatgagggacccagccctgggccgccgctgtggctgtgtgctggtggagtcagaatgtgtgtgcaagcgtgagaaactcctaggggacgtgctgtgcctggtgcaccaccacagggacccctcggcagtcttggggaagtgtagtagctccatcaaggcagctctctgcaccggcttccacctagacgtgtgcaagactgtgcagtggttccggaacatgatgggcaatgcctgggcccttgtggcccacaagtatgactttaaactcagtctcccaccgtctaccacctcctgcaagctccggctggactatcgctcaggccgctttctctcaatccacttggtcctgggggtgcaacgagaagacaccttggtctacctggtgagtcaggctcctgaccaggagcagctcaccagtgtggactggcctgagtcctttgtggcctgtgagcacctgttcctgaagctggtggggcgctttgcccccgagaacacctgtcacctcaagtgcctccagatcattttaagtctccggcagcatcagagcttaccccatggagcatcccgccccatcctcacttcttaccattttaaaacagctctcatgcacctcttgctacggctgcccctcacggactgggcccacaacatgctctctcagcggctccaggacattctctggttcttgggccgtggcctccagcaaaggtccctccatcatttcctcattggtaacaattttctgcccctgaccatcccaatccctaagacatttaggaatgctgagccggtcaatctcttccaacacctggtgctcaaccccaaggcacattcacaggcagtggaagagttccaaaaccttctgacccaggtgaaaactctgcctcatgccccactggctgcagcacctgattacaaggatgacgacgataagtgactcgag

SEQ ID NO: 9 - DNA, 237 bp, Homo sapiens
  source 1..237: mol_type = genomic DNA
cacccactgatggtgagcgaccgcatggacctcgacacactcgcccggtcacgacagctagaaaagcggatgtctgaggagatgagactgctggagatggagttcgaggagcgcaagcgcgccgccgagcagaggcagaaggccgagaacttctggaccggcgacacatcctctgaccagctcgtgctcggcaagaaggacatgggctggcctttccaggccgacggccaggagggc

SEQ ID NO: 10 - DNA, 162 bp, Homo sapiens
  source 1..162: mol_type = genomic DNA
gaccgcatggacctcgacacactcgcccggtcacgacagctagaaaagcggatgtctgaggagatgagactgctggagatggagttcgaggagcgcaagcgcgccgccgagcagaggcagaaggccgagaacttctggaccggcgacacatcctctgaccag

SEQ ID NO: 11 - DNA, 20 bp, synthetic construct
  misc_feature 1..20: note = synthetic oligonucleotide
  source 1..20: mol_type = other DNA
ccccagcactaactggtcac

SEQ ID NO: 12 - DNA, 20 bp, synthetic construct
  misc_feature 1..20: note = synthetic oligonucleotide
  source 1..20: mol_type = other DNA
agacatggggtggccgttcc

SEQ ID NO: 13 - DNA, 20 bp, synthetic construct
  misc_feature 1..20: note = synthetic oligonucleotide
  source 1..20: mol_type = other DNA
tcctggccatcggcctggaa

SEQ ID NO: 14 - DNA, 25 bp, synthetic construct
  misc_feature 1..25: note = synthetic oligonucleotide
  source 1..25: mol_type = other DNA
caccgccccagcactaactggtcac

SEQ ID NO: 15 - DNA, 25 bp, synthetic construct
  misc_feature 1..25: note = synthetic oligonucleotide
  source 1..25: mol_type = other DNA
aaacgtgaccagttagtgctggggc

SEQ ID NO: 16 - DNA, 25 bp, synthetic construct
  misc_feature 1..25: note = synthetic oligonucleotide
  source 1..25: mol_type = other DNA
caccgagacatggggtggccgttcc

SEQ ID NO: 17 - DNA, 25 bp, synthetic construct
  misc_feature 1..25: note = synthetic oligonucleotide
  source 1..25: mol_type = other DNA
aaacggaacggccaccccatgtctc

SEQ ID NO: 18 - DNA, 25 bp, synthetic construct
  misc_feature 1..25: note = synthetic oligonucleotide
  source 1..25: mol_type = other DNA
caccgtcctggccatcggcctggaa

SEQ ID NO: 19 - DNA, 25 bp, synthetic construct
  misc_feature 1..25: note = synthetic oligonucleotide
  source 1..25: mol_type = other DNA
aaacttccaggccgatggccaggac

SEQ ID NO: 20 - protein, 538 aa, synthetic construct
  REGION 1..538: note = synthetic peptide
HPLMVSDRMDLDTLARSRQLEKRMSEEMRLLEMEFEERKRAAEQRQKAENFWTGDTSSDQLVLGKKDMGWPFQADGQEGPLGWMLGNLWNTGLFCLFLVFELLRQNMQHEPAFDSSSEEEEEEVRVVPVTSYNWLTDFPSQEALDSFYKHYVQNAIRDLPCTCEFVESFVDDLIEACRVLSRQEAHPQLEDCLGIGAAFEKWGTLHETQKFDILVPIVPPQGTMFVLEMRDPALGRRCGCVLVESECVCKREKLLGDVLCLVHHHRDPSAVLGKCSSSIKAALCTGFHLDVCKTVQWFRNMMGNAWALVAHKYDFKLSLPPSTTSCKLRLDYRSGRFLSIHLVLGVQREDTLVYLVSQAPDQEQLTSVDWPESFVACEHLFLKLVGRFAPENTCHLKCLQIILSLRQHQSLPHGASRPILTSYHFKTALMHLLLRLPLTDWAHNMLSQRLQDILWFLGRGLQQRSLHHFLIGNNFLPLTIPIPKTFRNAEPVNLFQHLVLNPKAHSQAVEEFQNLLTQVKTLPHAPLAAAPDYKDDDK

SEQ ID NO: 21 - protein, 310 aa, synthetic construct; identical to SEQ ID NO: 5
  REGION 1..310: note = synthetic peptide

SEQ ID NO: 22 - protein, 461 aa, synthetic construct
  REGION 1..461: note = synthetic peptide
MEWRIFLFILSGTAGVHSQVQLQQSGPELVKPGASVRMSCKTSGYTFTDYVISWVKQRPGQGLEWIGEIFPRTGSTYYNENFKATATLTADKSSNTAYMQLSSLTSEDSAAYFCAFITSVDWAMEYWGQGTSVTVSSAKTTPPSVYPLAPGSAAQTNSMVTLGCLVKGYFPEPVTVTWNSGSLSSGVHTFPAVLQSDLYTLSSSVTVPSSTWPSETVTCNVAHPASSTKVDKKIVPRDCGCKPCICTVPEVSSVFIFPPKPKDVLTITLTPKVTCVVVDISKDDPEVQFSWFVDDVEVHTAQTQPREEQFNSTFRSVSELPIMHQDWLNGKEFKCRVNSAAFPAPIEKTISKTKGRPKAPQVYTIPPPKEQMAKDKVSLTCMITDFFPEDITVEWQWNGQPAENYKNTQPIMDTDGSYFVYSKLNVQKSNWEAGNTFTCSVLHEGLHNHHTEKSLSHSPGK

SEQ ID NO: 23 - protein, 238 aa, synthetic construct
  REGION 1..238: note = synthetic peptide
MKLPVRLLVLMFWIPGSSSDVVMTQTPLSLPVSLGDQASISCRSSESLVNSKGNTHLHWYLQKPGQSPKLLIYKVSNRFSGVPDRFSGSGSGTDFTLKISRVEAEDLGVYFCSQSTHAPYTFGGGTKLEIKRADAAPTVSIFPPSSEQLTSGGASVVCFLNNFYPKDINVKWKIDGSERQNGVLNSWTDQDSKDSTYSMSSTLTLTKDEYERHNSYTCEATHKTSTSPIVKSFNRNEC

SEQ ID NO: 24 - protein, 119 aa, synthetic construct
  REGION 1..119: note = synthetic peptide
QVQLQQSGPELVKPGASVRMSCKTSGYTFTDYVISWVKQRPGQGLEWIGEIFPRTGSTYYNENFKATATLTADKSSNTAYMQLSSLTSEDSAAYFCAFITSVDWAMEYWGQGTSVTVSS

SEQ ID NO: 25 - protein, 113 aa, synthetic construct
  REGION 1..113: note = synthetic peptide
DVVMTQTPLSLPVSLGDQASISCRSSESLVNSKGNTHLHWYLQKPGQSPKLLIYKVSNRFSGVPDRFSGSGSGTDFTLKISRVEAEDLGVYFCSQSTHAPYTFGGGTKLEIKR

SEQ ID NO: 26 - protein, 8 aa, synthetic construct
  REGION 1..8: note = synthetic peptide
GYTFTDYV

SEQ ID NO: 27 - protein, 8 aa, synthetic construct
  REGION 1..8: note = synthetic peptide
IFPRTGST

SEQ ID NO: 28 - protein, 12 aa, synthetic construct
  REGION 1..12: note = synthetic peptide
AFITSVDWAMEY

SEQ ID NO: 29 - protein, 11 aa, synthetic construct
  REGION 1..11: note = synthetic peptide
ESLVNSKGNTH

SEQ ID NO: 30 - skipped

SEQ ID NO: 31 - protein, 9 aa, synthetic construct
  REGION 1..9: note = synthetic peptide
SQSTHAPYT

SEQ ID NO: 32 - protein, 461 aa, synthetic construct
  REGION 1..461: note = synthetic peptide
MEWRIFLFILSGTAGVHSQVQLQQSGPELVKPGASVKMSCKASGYTFTDYVISWVKQRTGQGLEWIGEIFPRTGSTYFNENFKAKATLTADKSSNTAYMQLSSLTSEDSAAYFCAFITSVDWAMEYWGQGTSVTVSSAKTTPPSVYPLAPGSAAQTNSMVTLGCLVKGYFPEPVTVTWNSGSLSSGVHTFPAVLQSDLYTLSSSVTVPSSTWPSETVTCNVAHPASSTKVDKKIVPRDCGCKPCICTVPEVSSVFIFPPKPKDVLTITLTPKVTCVVVDISKDDPEVQFSWFVDDVEVHTAQTQPREEQFNSTFRSVSELPIMHQDWLNGKEFKCRVNSAAFPAPIEKTISKTKGRPKAPQVYTIPPPKEQMAKDKVSLTCMITDFFPEDITVEWQWNGQPAENYKNTQPIMDTDGSYFVYSKLNVQKSNWEAGNTFTCSVLHEGLHNHHTEKSLSHSPGK

SEQ ID NO: 33 - protein, 238 aa, synthetic construct
  REGION 1..238: note = synthetic peptide
MKLPVRLLVLMFWIPASSSDVVMTQIPLSLPVSLGDQASISCRSSQSLANSKGNTHLHWYLQKPGQSPKLLIYKVSNRFSGVPDRFSGSGSGTDFTLKISRVEAEDLGLYFCSQSTHVPYTFGGGTKLEIKRADAAPTVSIFPPSSEQLTSGGASVVCFLNNFYPKDINVKWKIDGSERQNGVLNSWTDQDSKDSTYSMSSTLTLTKDEYERHNSYTCEATHKTSTSPIVKSFNRNEC

SEQ ID NO: 34 - protein, 119 aa, synthetic construct
  REGION 1..119: note = synthetic peptide
QVQLQQSGPELVKPGASVKMSCKASGYTFTDYVISWVKQRTGQGLEWIGEIFPRTGSTYFNENFKAKATLTADKSSNTAYMQLSSLTSEDSAAYFCAFITSVDWAMEYWGQGTSVTVSS

SEQ ID NO: 35 - protein, 114 aa, synthetic construct
  REGION 1..114: note = synthetic peptide
DVVMTQIPLSLPVSLGDQASISCRSSQSLANSKGNTHLHWYLQKPGQSPKLLIYKVSNRFSGVPDRFSGSGSGTDFTLKISRVEAEDLGLYFCSQSTHVPYTFGGGTKLEIKRA

SEQ ID NO: 36 - protein, 8 aa, synthetic construct
  REGION 1..8: note = synthetic peptide
GYTFTDYV

SEQ ID NO: 37 - protein, 8 aa, synthetic construct
  REGION 1..8: note = synthetic peptide
IFPRTGST

SEQ ID NO: 38 - protein, 12 aa, synthetic construct
  REGION 1..12: note = synthetic peptide
AFITSVDWAMEY

SEQ ID NO: 39 - protein, 11 aa, synthetic construct
  REGION 1..11: note = synthetic peptide
QSLANSKGNTH

SEQ ID NO: 40 - skipped

SEQ ID NO: 41 - protein, 9 aa, synthetic construct
  REGION 1..9: note = synthetic peptide
SQSTHVPYT

SEQ ID NO: 42 - protein, 15 aa, synthetic construct
  REGION 1..15: note = synthetic peptide
HPLMVSDRMDLDTLA

SEQ ID NO: 43 - protein, 15 aa, synthetic construct
  REGION 1..15: note = synthetic peptide
VSDRMDLDTLARSRQ

SEQ ID NO: 44 - protein, 15 aa, synthetic construct
  REGION 1..15: note = synthetic peptide
MDLDTLARSRQLEKR

SEQ ID NO: 45 - protein, 15 aa, synthetic construct
  REGION 1..15: note = synthetic peptide
TLARSRQLEKRMSEE

SEQ ID NO: 46 - protein, 15 aa, synthetic construct
  REGION 1..15: note = synthetic peptide
SRQLEKRMSEEMRLL

SEQ ID NO: 47 - protein, 15 aa, synthetic construct
  REGION 1..15: note = synthetic peptide
EKRMSEEMRLLEMEF

SEQ ID NO: 48 - protein, 15 aa, synthetic construct
  REGION 1..15: note = synthetic peptide
SEEMRLLEMEFEERK

SEQ ID NO: 49 - protein, 15 aa, synthetic construct
  REGION 1..15: note = synthetic peptide
RLLEMEFEERKRAAE

SEQ ID NO: 50 - protein, 15 aa, synthetic construct
  REGION 1..15: note = synthetic peptide
MEFEERKRAAEQRQK

SEQ ID NO: 51 - protein, 15 aa, synthetic construct
  REGION 1..15: note = synthetic peptide
ERKRAAEQRQKAENF

SEQ ID NO: 52 - protein, 15 aa, synthetic construct
  REGION 1..15: note = synthetic peptide
AAEQRQKAENFWTGD

SEQ ID NO: 53 - protein, 15 aa, synthetic construct
  REGION 1..15: note = synthetic peptide
RQKAENFWTGDTSSD

SEQ ID NO: 54 - protein, 15 aa, synthetic construct
  REGION 1..15: note = synthetic peptide
ENFWTGDTSSDQLVL

SEQ ID NO: 55 - protein, 15 aa, synthetic construct
  REGION 1..15: note = synthetic peptide
TGDTSSDQLVLGKKD

SEQ ID NO: 56 - protein, 15 aa, synthetic construct
  REGION 1..15: note = synthetic peptide
SSDQLVLGKKDMGWP

SEQ ID NO: 57 - protein, 15 aa, synthetic construct
  REGION 1..15: note = synthetic peptide
LVLGKKDMGWPFQAD

SEQ ID NO: 58 - protein, 15 aa, synthetic construct
  REGION 1..15: note = synthetic peptide
KKDMGWPFQADGQEG

SEQ ID NO: 59 - protein, 15 aa, synthetic construct
  REGION 1..15: note = synthetic peptide
ALLEMEFEERKRAAE

SEQ ID NO: 60 - protein, 15 aa, synthetic construct
  REGION 1..15: note = synthetic peptide
RALEMEFEERKRAAE

SEQ ID NO: 61 - protein, 15 aa, synthetic construct
  REGION 1..15: note = synthetic peptide
RLAEMEFEERKRAAE

SEQ ID NO: 62 - protein, 15 aa, synthetic construct
  REGION 1..15: note = synthetic peptide
RLLAMEFEERKRAAE

SEQ ID NO: 63 - protein, 15 aa, synthetic construct
  REGION 1..15: note = synthetic peptide
RLLEAEFEERKRAAE

SEQ ID NO: 64 - protein, 15 aa, synthetic construct
  REGION 1..15: note = synthetic peptide
RLLEMAFEERKRAAE

SEQ ID NO: 65 - protein, 15 aa, synthetic construct
  REGION 1..15: note = synthetic peptide
RLLEMEAEERKRAAE

SEQ ID NO: 66 - protein, 15 aa, synthetic construct
  REGION 1..15: note = synthetic peptide
RLLEMEFAERKRAAE

SEQ ID NO: 67 - protein, 15 aa, synthetic construct
  REGION 1..15: note = synthetic peptide
RLLEMEFEARKRAAE

SEQ ID NO: 68 - protein, 15 aa, synthetic construct
  REGION 1..15: note = synthetic peptide
RLLEMEFEEAKRAAE

SEQ ID NO: 69 - protein, 15 aa, synthetic construct
  REGION 1..15: note = synthetic peptide
RLLEMEFEERARAAE

SEQ ID NO: 70 - protein, 15 aa, synthetic construct
  REGION 1..15: note = synthetic peptide
RLLEMEFEERKAAAE

SEQ ID NO: 71 - protein, 15 aa, synthetic construct
  REGION 1..15: note = synthetic peptide
RLLEMEFEERKRAAA

SEQ ID NO: 72 - protein, 15 aa, synthetic construct
  REGION 1..15: note = synthetic peptide
RLLEMEFEERKQAAE

SEQ ID NO: 73 - protein, 119 aa, synthetic construct
  REGION 1..119: note = synthetic peptide
QVQLQESGPGLVKPSETLSLTCTTSGYTFTDYVISWVRQPPGKGLEWIGEIFPRTGSTYYNENFKARATLSADKSKNQASLNLDSVSAADTAIYFCAFITSVDWAMEYWGKGSTVTVSS

SEQ ID NO: 74 - protein, 113 aa, synthetic construct
  REGION 1..113: note = synthetic peptide
DIQMTQSPSSLSASVGDRVTITCRSSESLVNSKGNTHLHWYQQKPGKAPKLLIYKVSNRFSGVPSRFSGSGSGTDFTFTISSLQPEDIATYFCSQSTHAPYTFGPGTKVDIKR

SEQ ID NO: 75 - protein, 116 aa, synthetic construct
  REGION 1..116: note = synthetic peptide
QVQLVQSGAEVKKPGASVKVSCKTSGYTFTDYVISWVRQAPGQGLEWIGEIFPRTGSTYYNENFKAKATLTADKSTSTAYMELSSLRSEDTAVYFCAFITSVDWAMEYWGQGTLVT

SEQ ID NO: 76 - protein, 113 aa, synthetic construct
  REGION 1..113: note = synthetic peptide
DVVMTQTPLSLSVTPGQPASISCRSSESLVNSKGNTHLHWYLQKPGQSPKLLIYKVSNRFSGVPDRFSGSGSGTGFTLKISRVEAEDVGVYFCSQSTHAPYTFGGGTKLEIKR

SEQ ID NO: 77 - protein, 119 aa, synthetic construct
  REGION 1..119: note = synthetic peptide
EVQLVQSGAEVKKPGESLKISCQTFGYTFTDYVISWVRQMPGQGLEWIGEIFPRTGSTYYNENFKAQATLSADKSSSTAYLQWSSLKASDTAMYFCAFITSVDWAMEYWGQGTMVTVSS

SEQ ID NO: 78 - protein, 113 aa, synthetic construct
  REGION 1..113: note = synthetic peptide
DVVMTQTPLSLPVTPGEPASISCRSSESLVNSKGNTHLHWYLQKPGQSPKLLIYKVSNRFSGVPDRFSGSGSGTDFTLKISRVEAEDVGVYFCSQSTHAPYTFGQGTKLEIKR

SEQ ID NO: 79 - protein, 119 aa, synthetic construct
  REGION 1..119: note = synthetic peptide
EVTLKESGPVLVKPTETLTLTCTTSGYTFTDYVISWVRQPPGKALEWIGEIFPRTGSTYYNENFKARATLSADKSKSQAVLTMTNMDPVDTATYFCAFITSVDWAMEYWGQGTLVTVSS

SEQ ID NO: 80 - protein, 113 aa, synthetic construct
  REGION 1..113: note = synthetic peptide
EVVMTQSPATLSLSPGERATLSCRSSESLVNSKGNTHLHWYQQKPGQAPRLLIYKVSNRFSGIPARFSGSGSGTDFTLTISSLEPEDFAVYFCSQSTHAPYTFGQGTKLEIKR

SEQ ID NO: 81 - protein, 119 aa, synthetic construct
  REGION 1..119: note = synthetic peptide
EVQLVESGGGLVQPGGSLRLSCATSGYTFTDYVISWVRQAPGKGLEWIGEIFPRTGSTYYNENFKARATLSADKSKNTAYLQMNSLRAEDTAVYFCAFITSVDWAMEYWGQGTLVTVSS

SEQ ID NO: 82 - protein, 113 aa, synthetic construct
  REGION 1..113: note = synthetic peptide
DVQMTQSPSSLSASVGDRVTITCRSSESLVNSKGNTHLHWYQQKPGKAPKLLIYKVSNRFSGVPSRFSGSGSGTDFTLTISSLQPEDFATYFCSQSTHAPYTFGQGTKVEIKR

SEQ ID NO: 83 - protein, 54 aa, synthetic construct
  REGION 1..54: note = RBD1 derivative sequence
  SITE 24: note = MISC_FEATURE - "Xaa" is any amino acid
  REGION 33..35: note = MISC_FEATURE - "Xaa" is any amino acid
  REGION 38..39: note = MISC_FEATURE - "Xaa" is any amino acid
  SITE 42: note = MISC_FEATURE - "Xaa" is any amino acid
  SITE 45: note = MISC_FEATURE - "Xaa" is any amino acid
  SITE 47: note = MISC_FEATURE - "Xaa" is any amino acid
  SITE 49: note = MISC_FEATURE - "Xaa" is any amino acid
  SITE 52: note = MISC_FEATURE - "Xaa" is any amino acid
DRMDLDTLARSRQLEKRMSEEMRXLEMEFEERXXXAEXXQKXENXWXGXTSXDQ

SEQ ID NO: 84 - skipped

SEQ ID NO: 85 - protein, 231 aa, synthetic construct
  REGION 1..231: note = Fc without CH1
PKSCDKTHTCPPCPAPELLGGPSVFLFPPKPKDTLMISRTPEVTCVVVDVSHEDPEVKFNWYVDGVEVHNAKTKPREEQYNSTYRVVSVLTVLHQDWLNGKEYKCKVSNKALPAPIEKTISKAKGQPREPQVYTLPPSRDELTKNQVSLTCLVKGFYPSDIAVEWESNGQPENNYKTTPPVLDSDGSFFLYSKLTVDKSRWQQGNVFSCSVMHEALHNHYTQKSLSLSPGK

SEQ ID NO: 86 - DNA, 44 bp, synthetic construct
  misc_feature 1..44: note = Sequence displayed in Fig1
  source 1..44: mol_type = other DNA
taagcctgctgttcttggcagtgatgtatgttgttcaccaccct

SEQ ID NO: 87 - DNA, 27 bp, synthetic construct
  misc_feature 1..27: note = Sequence displayed in Fig4
  source 1..27: mol_type = other DNA
catggacctcgacacactcgcccggtc

SEQ ID NO: 88 - protein, 26 aa, synthetic construct
  REGION 1..26: note = secondary structure predicition, ITPRIPL1
HHHHHHHHHHHHHHHHHHHHHHHHHH

SEQ ID NO: 89 - protein, 42 aa, synthetic construct
  REGION 1..42: note = secondary structure predicition, ITPRIPL1
HHHHHHHHHHHHHHHHHHHHHHHHHHHHHHHHHHHHHHHHHH

SEQ ID NO: 90 - protein, 96 aa, Mus musculus
MAVISLMFLAVMYVVHHPLMVSDRMDLDTLARSRQLEKRMSEEMRQLEMEFEERSRAAEQKQKVENFWRGDTSSDQLVLGKKDMGWPFQAGGQDGG

SEQ ID NO: 91 - protein, 96 aa, Rattus norvegicus
MAVISLLFLAVMYVVHHPLMVSDRMDLDTLARSRQLEKRMSEEMRQLEIEFEERSRAAEEKQKAENFWRGDTSNDQLVLGKKDMRWPFQASGQDGG

SEQ ID NO: 92 - protein, 103 aa, Pan troglodytes; identical to SEQ ID NO: 4
  REGION 1..103: note = MISC_FEATURE - H2QIC9 PANTR

SEQ ID NO: 93 - protein, 103 aa, Chlorocebus sabaeus
  REGION 1..103: note = MISC_FEATURE - A0A0D9RXR0_CHLSB
MNLDAEASMAVISLLFLAVMYVVHHPLMVSDRMDLDTLARSRQLEKRMSEEMRLLEMEFEERKQAAEQKQKAENFWRGDTSSDQLVLGKKDTGWPLQADGQEG

SEQ ID NO: 94 - protein, 103 aa, Rhinopithecus roxellana
  REGION 1..103: note = MISC_FEATURE - A0A2K6PNR9_RHIRO
MNLDAEASMAVISLLFLAVMYVVHHPLMVSDRMDLDTLARSRQLEKRMSEEMRLLEMEFEERKQAAEQKQKAENLWRGDTSSDQLVLGKKDMGWPFQADGQEG

SEQ ID NO: 95 - protein, 103 aa, Rhinopithecus bieti; identical to SEQ ID NO: 94
  REGION 1..103: note = MISC_FEATURE - A0A2K6KJX9_RHIBE

SEQ ID NO: 96 - protein, 103 aa, Saimiri boliviensis
  REGION 1..103: note = MISC_FEATURE - A0A2K6TF56_SAIBB
MNLDAEASMAVISLLFLAVMYVVHHPLMVSDRMDLDTLARSRQLEKRMSEEMRLLEMEFEERKRAAEQKQKAENFWRGETSSDQLVLGKKDMGWPFQDDAQEG

SEQ ID NO: 97 - protein, 103 aa, Aotus nancymai
  REGION 1..103: note = MISC_FEATURE - A0A2K5E6W3_AOTNA
MNLDAAASMAVISLLFLAVMYVVQNPLMVSDRMDLDTLARSRQLEKRMSEEMRLLEMEFEERKRVAEQKQKAENFWRGDTSSDQLVLGKKDMRWPFQADGQEG

SEQ ID NO: 98 - protein, 11 aa, synthetic construct
  REGION 1..11: note = LCDR1
  SITE 1: note = MISC_FEATURE - "Xaa" is any amino acid
  SITE 4: note = MISC_FEATURE - "Xaa" is any amino acid
XSLXNSKGNTH

SEQ ID NO: 99 - protein, 9 aa, synthetic construct
  REGION 1..9: note = LCDR3
  SITE 6: note = MISC_FEATURE - "Xaa" is any amino acid
SQSTHXPYT